European Patent Application EP 4 276 105 A1, published November 15, 2023. Title: POLYPEPTIDE FOR REPAIRING SKIN WOUND OR MUCOSAL INJURY, AND APPLICATION THEREOF. Applicant: SICHUAN GOODDOCTOR PANXI PHARMACEUTICAL CO., LTD. Application EP21917328.3. The sequence listing filed with the application follows.

SEQUENCE LISTING (73 sequences)

SEQ ID NO: 1 - protein, 15 aa, Artificial Sequence
SMQASLEAEAKGKAE

SEQ ID NO: 2 - protein, 13 aa, Artificial Sequence
QASLEAEAKGKAE

SEQ ID NO: 3 - protein, 13 aa, Artificial Sequence
SMQASLEAEAKGK

SEQ ID NO: 4 - protein, 11 aa, Artificial Sequence
QASLEAEAKGK

SEQ ID NO: 5 - protein, 11 aa, Artificial Sequence
SMQASLEAEAK

SEQ ID NO: 6 - protein, 9 aa, Artificial Sequence
QASLEAEAK

SEQ ID NO: 7 - protein, 9 aa, Artificial Sequence
EAEAKGKAE

SEQ ID NO: 8 - protein, 6 aa, Artificial Sequence
SMQASL

SEQ ID NO: 9 - protein, 4 aa, Artificial Sequence
QASL

SEQ ID NO: 10 - protein, 4 aa, Artificial Sequence
GKAE

SEQ ID NO: 11 - protein, 15 aa, Artificial Sequence
SMQASLEAEAKGKAE

SEQ ID NO: 12 - protein, 15 aa, Artificial Sequence
SVQASLEAEAKGKAE

SEQ ID NO: 13 - protein, 15 aa, Artificial Sequence
SMQASLEAEAKGKAQ

SEQ ID NO: 14 - protein, 15 aa, Artificial Sequence
SMQASLQAQAKGKAE

SEQ ID NO: 15 - protein, 15 aa, Artificial Sequence
SMQASAEAEAKGKAE

SEQ ID NO: 16 - protein, 15 aa, Artificial Sequence
SAQASLEAEAKGKAE

SEQ ID NO: 17 - protein, 15 aa, Artificial Sequence
SLQASLEAEAKGKAE

SEQ ID NO: 18 - protein, 15 aa, Artificial Sequence
SMQASLEAEAAGKAE

SEQ ID NO: 19 - protein, 15 aa, Artificial Sequence
SMQASLAAEAKGKAE

SEQ ID NO: 20 - protein, 15 aa, Artificial Sequence
SMQASLEAAAKGKAE

SEQ ID NO: 21 - protein, 15 aa, Artificial Sequence
SMAASLEAEAKGKAE

SEQ ID NO: 22 - protein, 15 aa, Artificial Sequence
SIQASLEAEAKGKAE

SEQ ID NO: 23 - protein, 15 aa, Artificial Sequence
SMQASLEAEAKGKAD

SEQ ID NO: 24 - protein, 15 aa, Artificial Sequence
SMQASLEAEAKGKAN

SEQ ID NO: 25 - protein, 15 aa, Artificial Sequence
SMQASLEAEAKGRAE

SEQ ID NO: 26 - protein, 15 aa, Artificial Sequence
SMQASLEAEAKGAAE

SEQ ID NO: 27 - protein, 15 aa, Artificial Sequence
SMQASLEAEAKGKAA

SEQ ID NO: 28 - protein, 15 aa, Artificial Sequence
SMQAALEAEAKGKAE

SEQ ID NO: 29 - protein, 15 aa, Artificial Sequence
AMQASLEAEAKGKAE

SEQ ID NO: 30 - protein, 15 aa, Artificial Sequence
SMQASLEAEARGKAE

SEQ ID NO: 31 - protein, 15 aa, Artificial Sequence
SMQASLEAEAKGHAE

SEQ ID NO: 32 - protein, 15 aa, Artificial Sequence
SMQASLEAEAHGKAE

SEQ ID NO: 33 - protein, 15 aa, Artificial Sequence
SMQASLLAEAKGKAE

SEQ ID NO: 34 - protein, 15 aa, Artificial Sequence
SMQASLEALAKGKAE

SEQ ID NO: 35 - protein, 15 aa, Artificial Sequence
SMQASLQAEAKGKAE

SEQ ID NO: 36 - protein, 15 aa, Artificial Sequence
SMQASLEAQAKGKAE

SEQ ID NO: 37 - protein, 15 aa, Artificial Sequence
SMEASLEAEAKGKAE

SEQ ID NO: 38 - protein, 15 aa, Artificial Sequence
SMQASLDAEAKGKAE

SEQ ID NO: 39 - protein, 15 aa, Artificial Sequence
SMQASLEADAKGKAE

SEQ ID NO: 40 - protein, 15 aa, Artificial Sequence
TMQASLEAEAKGKAE

SEQ ID NO: 41 - protein, 15 aa, Artificial Sequence
SMQATLEAEAKGKAE

SEQ ID NO: 42 - protein, 15 aa, Artificial Sequence
SMQASVEAEAKGKAE

SEQ ID NO: 43 - protein, 15 aa, Artificial Sequence
SMQASLESEAKGKAE

SEQ ID NO: 44 - protein, 15 aa, Artificial Sequence
SMQASLEAESKGKAE

SEQ ID NO: 45 - protein, 4 aa, Artificial Sequence
EAEA

SEQ ID NO: 46 - protein, 7 aa, Artificial Sequence
EAEAKGK

SEQ ID NO: 47 - protein, 14 aa, Artificial Sequence
TASTLEAEAKGKAE

SEQ ID NO: 48 - protein, 15 aa, Artificial Sequence
STQASLEAEAKGKAE

SEQ ID NO: 49 - protein, 16 aa, Artificial Sequence
SMQASLEAEAKGKAQD

SEQ ID NO: 50 - protein, 16 aa, Artificial Sequence
SMQASLEAEAKGKAQE

SEQ ID NO: 51 - protein, 16 aa, Artificial Sequence
SMQASLEAEAKGKAEL

SEQ ID NO: 52 - protein, 16 aa, Artificial Sequence
SMQASLEAEAKGKAEA

SEQ ID NO: 53 - protein, 17 aa, Artificial Sequence
SMQASLEAEAKGKAKQD

SEQ ID NO: 54 - protein, 15 aa, Artificial Sequence
AEPVPLEAEAKGKAE

SEQ ID NO: 55 - protein, 17 aa, Artificial Sequence
PAAEPVPLEAEAKGKAE

SEQ ID NO: 56 - protein, 15 aa, Artificial Sequence
SMQASLEAEAKAKAE

SEQ ID NO: 57 - protein, 15 aa, Artificial Sequence
SMQASLEAEAKPKAE

SEQ ID NO: 58 - protein, 17 aa, Artificial Sequence
SMQASLEAEAKGKAKQE

SEQ ID NO: 59 - protein, 14 aa, Artificial Sequence
RKDVYEAEAKGKAE

SEQ ID NO: 60 - protein, 15 aa, Artificial Sequence
SMQASLEAEAKGKSE

SEQ ID NO: 61 - protein, 9 aa, Artificial Sequence
EAEAAGKAE

SEQ ID NO: 62 - protein, 14 aa, Artificial Sequence
FDALKQQFQAFQLE

SEQ ID NO: 63 - protein, 14 aa, Artificial Sequence
HCLAGLKKDLEDLE

SEQ ID NO: 64 - protein, 13 aa, Artificial Sequence
EINQLELIKQASI

SEQ ID NO: 65 - protein, 11 aa, Artificial Sequence
AARLADELRAE

SEQ ID NO: 66 - protein, 9 aa, Artificial Sequence
ETLQRKNKE

SEQ ID NO: 67 - protein, 10 aa, Artificial Sequence
VDAAVLEKLE

SEQ ID NO: 68 - protein, 8 aa, Artificial Sequence
AAVLDKLE

SEQ ID NO: 69 - protein, 8 aa, Artificial Sequence
AAVLEKLE

SEQ ID NO: 70 - protein, 28 aa, Artificial Sequence
KFYSQSTASSSYAYPSHFGPAGFSGSHS

SEQ ID NO: 71 - protein, 10 aa, Artificial Sequence
VDAAVIEKIE

SEQ ID NO: 72 - protein, 10 aa, Artificial Sequence
VDAAMVLLTR

SEQ ID NO: 73 - protein, 10 aa, Artificial Sequence
VDAAVLMLRT